European Patent Application EP 4 374 845 A1, published May 29, 2024. Title: COMPOSITION COMPRISING SUPEROXIDE DISMUTASE AND/OR BACILLUS STRAIN SPORES, AND USES THEREOF FOR IMPROVING ORAL HEALTH. Applicant: GENOFOCUS CO., LTD. The sequence listing filed with the application follows.

SEQUENCE LISTING (4 sequences)

SEQ ID NO: 1 - DNA, 606 bp, Bacillus amyloliquefaciens
  source 1..606: mol_type = other DNA
atggcttacaaacttccagaattgccttacgcttatgatgctttagaacctcatatcgataaggaaacgatgacgattcaccatacgaagcaccataacacatacgtgacaaacctcaacaaagcgatcgaaggatctgcgcttgcagagaaatctgtagatgagcttgttgctgatttgaacgcagtgccggaggacatccgcacggcagtccgcaacaatggcggcggacatgcaaaccactctttattctggactcttttatctccgaacggcggaggcgaaccgactggtgagcttgctgaagagatcaaaagcacgttcggaagcttcgatcaatttaaagaaaaattcgccgcagcagctgcaggccgtttcggttcaggctgggcttggctcgttgtaaacaacggcaaacttgaaattacaagcacgccaaaccaagattcaccgctttcagaaggtaaaacacctgttctcggtcttgatgtttgggagcatgcgtactacctgaactaccaaaaccgccgtcctgattacatttcagctttctggaatgttgtgaactgggatgaagttgcccgtctttacagcgaagcaaaataa

SEQ ID NO: 2 - protein, 201 aa, Bacillus amyloliquefaciens
MAYKLPELPYAYDALEPHIDKETMTIHHTKHHNTYVTNLNKAIEGSALAEKSVDELVADLNAVPEDIRTAVRNNGGGHANHSLFWTLLSPNGGGEPTGELAEEIKSTFGSFDQFKEKFAAAAAGRFGSGWAWLVVNNGKLEITSTPNQDSPLSEGKTPVLGLDVWEHAYYLNYQNRRPDYISAFWNVVNWDEVARLYSEAK

SEQ ID NO: 3 - DNA, 606 bp, Bacillus amyloliquefaciens
  source 1..606: mol_type = other DNA
atggcttacaaacttccagaattgccttacgcttatgatgctttagaacctcatatcgataaggaaacgatgacgattcaccatacgaagcaccataacacatacgtgacaaacctcaacaaagcgatcgaaggatctgcgcttgcagagaaatctgtagatgagcttgttgctgatttgaacgcagtgccggaggacatccgcacggcagtccgcaacgatggcggcggacatgcaaaccactctttattctggactcttttatctccgaacggcggaggcgaaccgactggtgagcttgctgaagagatcaaaagcacgttcggaagcttcgatcaatttaaagaaaaattcgccgcagcagctgcaggccgtttcggttcaggctgggcttggctcgttgtaaacgacggcaaacttgaaattacaagcacgccaaaccaagattcaccgctttcagaaggtaaaacacctgttctcggtcttgatgtttgggagcatgcgtactacctgaactaccaaaaccgccgtcctgattacatttcagctttctggaatgttgtgaactgggatgaagttgcccgtctttacagcgaagcaaaataa

SEQ ID NO: 4 - protein, 201 aa, Bacillus amyloliquefaciens
MAYKLPELPYAYDALEPHIDKETMTIHHTKHHNTYVTNLNKAIEGSALAEKSVDELVADLNAVPEDIRTAVRNDGGGHANHSLFWTLLSPNGGGEPTGELAEEIKSTFGSFDQFKEKFAAAAAGRFGSGWAWLVVNDGKLEITSTPNQDSPLSEGKTPVLGLDVWEHAYYLNYQNRRPDYISAFWNVVNWDEVARLYSEAK